European Patent Specification EP 3 630 178 B1, published May 14, 2025. Title: MMP13 Binding Immunoglobulins. Applicant: Merck Patent GmbH Ablynx N.V. The sequence listing filed with the application follows.

SEQUENCE LISTING (197 sequences)

SEQ ID NO: 1 - protein, 114 aa, Artificial Sequence
  Amino acid sequence
EVQLVESGGGSVQAGGSLRLSCAASGSTFSRYSMNWYRQAPGKQREFVAGISVGRITNYAVSVRGRFTISRDNAEGTGYLQMNSLKPEDTAVYYCNAGGLQGYWGLGTQVTVSS

SEQ ID NO: 2 - protein, 114 aa, Artificial Sequence
  Amino acid sequence
KVQLVESGGGSVQAGGSLRLSCAASGSTFSRRSMNWYRQAPGKQREFVAGISTGRITNYAVSVKGRFTISRDNAEGTGYLQMNSLKPEDTAVYYCNAGGLQGYWGLGTQVTVSS

SEQ ID NO: 3 - protein, 114 aa, Artificial Sequence
  Amino acid sequence
EVQLVESGRGSVQAGGSLRLSCAASGSTFSRRSMNWYRQAPGKQREFVAGISTGRITNYAVSVKGRFTISRDNAEGTGYLQMNSLKPEDTAVYYCNAGGLQGYWGLGTQVTVSS

SEQ ID NO: 4 - protein, 114 aa, Artificial Sequence
  Amino acid sequence
EVQLVESGGGSVQTGGSLRLSCAASGSTFSRRSMNWYRQAPGKQREFVAGISTGRITNYAVSVKGRFTISRDNAEGTGYLQMNSLKPEDTAVYYCNAGGLQGYWGLGTQVTVSS

SEQ ID NO: 5 - protein, 114 aa, Artificial Sequence
  Amino acid sequence
EVQLVESEGGSVQAGGSLRLSCAASGSTFSRYSMNWYRQAPGKQREFVAGISVGRITNYAVSVRGRFTISRDNAEGTGYLQMNSLKPEDTAVYYCNAGGLQGYWGLGTQVTVSS

SEQ ID NO: 6 - protein, 114 aa, Artificial Sequence
  Amino acid sequence
EVQLVESRGGSVQAGGSLRLSCAASGSTFSRYSMNWYRQAPGKQREFVAGISVGRITNYAVSVKGRFTISRDNAEGTGYLQMNSLKPEDTAVYYCNAGGLQGYWGLGTQVTVSS

SEQ ID NO: 7 - protein, 114 aa, Artificial Sequence
  Amino acid sequence
EVQLVESGGGSVQAGGSLRLSCAASGSTFSRYSMNWYRQAPGKQREFVAGISVGRITNYAVSVKGRFTISRDNAEGTGFLQMNGLKPEDTAVYYCNAGGLQGYWGLGTQVTVSS

SEQ ID NO: 8 - protein, 114 aa, Artificial Sequence
  Amino acid sequence
EVQLVESGGGSVQAGGSLRLSCAASGSTFSRYSMNWYRQAPRKQREFVAGISTARITHYAVSVKGRFTISRDNAEGTGYLQMNSLKPEDTAVYYCNAGGLQGSWGLGTLVTVSS

SEQ ID NO: 9 - protein, 123 aa, Artificial Sequence
  Amino acid sequence
DVQLVESGGGLVQPGGSLRLSCVASGSIFSINAMGWYRQAPGKQRELVAAISSGGSTYYADSVKGRFTISRDNSKNTVYLQMNSLRPEDTAVYYCNAAVDASRGLPYELYYYWGQGTLVTVSS

SEQ ID NO: 10 - protein, 129 aa, Artificial Sequence
  Amino acid sequence
DVQLVESGGGLVQPGGSLRLSCAASGRTFSSYAMGWFRQAPGKEREFVAAISWSGGSTYYADSVKGRFTISRDNSKNTVYLQMNSLRPEDTAVYYCTAALAVYGPNRYRYGPVGEYNYWGQGTLVTVSS

SEQ ID NO: 11 - protein, 121 aa, Artificial Sequence
  Amino acid sequence
EVQLVESGGALVRPGGSLRLSCAASGFAFSAAYMSWVRQAPGRGLEWVSSISDDGSKTYYADSVKGRFTISRDNAKNTVYLQMNNLKPDDTAVYYCNTGYGATTTRPGRYWGQGTQVTVSS

SEQ ID NO: 12 - protein, 128 aa, Artificial Sequence
  Amino acid sequence
EVQLVESGGGLVQPGGSLRLSCAASGFTLAYYSIGWFRQAPGKEREGVSCISSGIDGSTYYADSVKGRFTISRDNAKNTMYLQMNNLKPEDTGVYYCAADPSHYYSEYDCGYYGMDYWGKGTLVTVSS

SEQ ID NO: 13 - protein, 120 aa, Artificial Sequence
  Amino acid sequence
DVQLVESGGGLVQPGGSLRLSCAGSGSIFRINVMAWYRQAPGKQRELVAAITSGGTTNYADSVKGRFTISRDNSKNTVYLQMNSLRPEDTAVYYCYADIGWPYVLDYDFWGQGTLVTVSS

SEQ ID NO: 14 - protein, 120 aa, Artificial Sequence
  Amino acid sequence
DVQLVESGGGLVQPGGSLRLSCAASGSIFRINAMGWYRQAPGKQRELVAAIISGGTTYYADSVKGRFTISRDNSKNTVYLQMNSLRPEDTAVYYCYADIGWPYVLDYDFWGQGTLVTVSS

SEQ ID NO: 15 - protein, 126 aa, Artificial Sequence
  Amino acid sequence
DVQLVESGGGLVQPGGSLRLSCAASGRTFSRYVMGWFRQAPGKEREFVAAINWSSGSTYYADSVKGRFTISRDNSKNTVYLQMNSLRPEDTAVYYCAADRRVYYDTYPNLRGYDYWGQGTLVTVSS

SEQ ID NO: 16 - protein, 124 aa, Artificial Sequence
  Amino acid sequence
DVQLVESGGGLVQPGGSLRLSCVASGLTFSSYAMGWFRQAPGKEREFVAAISWSGGRTYYADSVKGRFTISRDNSKNTVYLQMNSLRPEDTAVYYCTAARGPGSVGPSEEYNYWGQGTLVTVSS

SEQ ID NO: 17 - protein, 127 aa, Artificial Sequence
  Amino acid sequence
DVQLVESGGGLVQPGGSLRLSCVASGPTFSDYAMGWFRQAPGKEREFVAAISWSGGSTYYADSVKGRFTISRDNSKNTVYLQMNSLRPEDTAVYYCTAARGGGYRASGGPLSEYNYWGQGTLVTVSS

SEQ ID NO: 18 - protein, 126 aa, Artificial Sequence
  Amino acid sequence
DVQLVESGGGLVQPGGSLRLSCAASGRTFSSYAMGWFRQAPGKEREFVAAISWGGGSTYYSDSVKGRFTISRDNSKNTVYLQMNSLRPEDTAVYYCTAALGSTGSGSTPVPEYRYWGQGTLVTVSS

SEQ ID NO: 19 - protein, 126 aa, Artificial Sequence
  Amino acid sequence
DVQLVESGGGLVQPGGSLRLSCAASGRTFSSYAMGWFRQAPGKEREFVAAISWSGGSTYYSDSVKGRFTISRDNSKNTVYLQMNSLRPEDTAVYYCTAARGGVAGTDGPLGDYNYWGQGTLVTVSS

SEQ ID NO: 20 - protein, 120 aa, Artificial Sequence
  Amino acid sequence
DVQLVESGGGLVQPGGSLRLSCAGSGSIFSGNAMGWYRQAPGKQRELVAAITSGGVTNYADSVKGRFTISRDNSKNTVYLQMNSLRPEDTAVYYCAADIRYPTGLVGDYWGQGTLVTVSS

SEQ ID NO: 21 - protein, 120 aa, Artificial Sequence
  Amino acid sequence
EVQLVESGGGLVQPGGSLRLSCSASTGIFRINTMGWHRQAPGKQRDLVATFTSDDNTKYADSVKGRFTISRDNAENTVYLQMNDLKPEDTAVYYCHATTVMYDSNSPDYWGQGTQVTVSS

SEQ ID NO: 22 - protein, 128 aa, Artificial Sequence
  Amino acid sequence
EVQLVESEGGTVEPGESLRLACAAPGPGIRTNFMAWYRQAPEKEREMVASISRDGSTHYADSVKGRFTISSDNATSTFYLQMNSLQVEDTAVYYCATDPHILHNDRAGAFLVEDYDHWGQGTQVTVSS

SEQ ID NO: 23 - protein, 10 aa, Artificial Sequence
  Amino acid sequence
GSTFSRYSMN

SEQ ID NO: 24 - protein, 10 aa, Artificial Sequence
  Amino acid sequence
GSTFSRRSMN

SEQ ID NO: 25 - protein, 10 aa, Artificial Sequence
  Amino acid sequence
GSIFSINAMG

SEQ ID NO: 26 - protein, 10 aa, Artificial Sequence
  Amino acid sequence
GRTFSSYAMG

SEQ ID NO: 27 - protein, 10 aa, Artificial Sequence
  Amino acid sequence
GFAFSAAYMS

SEQ ID NO: 28 - protein, 10 aa, Artificial Sequence
  Amino acid sequence
GFTLAYYSIG

SEQ ID NO: 29 - protein, 10 aa, Artificial Sequence
  Amino acid sequence
GSIFRINVMA

SEQ ID NO: 30 - protein, 10 aa, Artificial Sequence
  Amino acid sequence
GSIFRINAMG

SEQ ID NO: 31 - protein, 10 aa, Artificial Sequence
  Amino acid sequence
GRTFSRYVMG

SEQ ID NO: 32 - protein, 10 aa, Artificial Sequence
  Amino acid sequence
GLTFSSYAMG

SEQ ID NO: 33 - protein, 10 aa, Artificial Sequence
  Amino acid sequence
GPTFSDYAMG

SEQ ID NO: 34 - protein, 10 aa, Artificial Sequence
  Amino acid sequence
GSIFSGNAMG

SEQ ID NO: 35 - protein, 10 aa, Artificial Sequence
  Amino acid sequence
TGIFRINTMG

SEQ ID NO: 36 - protein, 10 aa, Artificial Sequence
  Amino acid sequence
GPGIRTNFMA

SEQ ID NO: 37 - protein, 9 aa, Artificial Sequence
  Amino acid sequence
GISVGRITN

SEQ ID NO: 38 - protein, 9 aa, Artificial Sequence
  Amino acid sequence
GISTGRITN

SEQ ID NO: 39 - protein, 9 aa, Artificial Sequence
  Amino acid sequence
GISTARITH

SEQ ID NO: 40 - protein, 9 aa, Artificial Sequence
  Amino acid sequence
AISSGGSTY

SEQ ID NO: 41 - protein, 10 aa, Artificial Sequence
  Amino acid sequence
AISWSGGSTY

SEQ ID NO: 42 - protein, 10 aa, Artificial Sequence
  Amino acid sequence
SISDDGSKTY

SEQ ID NO: 43 - protein, 11 aa, Artificial Sequence
  Amino acid sequence
CISSGIDGSTY

SEQ ID NO: 44 - protein, 9 aa, Artificial Sequence
  Amino acid sequence
AITSGGTTN

SEQ ID NO: 45 - protein, 9 aa, Artificial Sequence
  Amino acid sequence
AIISGGTTY

SEQ ID NO: 46 - protein, 10 aa, Artificial Sequence
  Amino acid sequence
AINWSSGSTY

SEQ ID NO: 47 - protein, 10 aa, Artificial Sequence
  Amino acid sequence
AISWSGGRTY

SEQ ID NO: 48 - protein, 10 aa, Artificial Sequence
  Amino acid sequence
AISWGGGSTY

SEQ ID NO: 49 - protein, 9 aa, Artificial Sequence
  Amino acid sequence
AITSGGVTN

SEQ ID NO: 50 - protein, 9 aa, Artificial Sequence
  Amino acid sequence
TFTSDDNTK

SEQ ID NO: 51 - protein, 9 aa, Artificial Sequence
  Amino acid sequence
SISRDGSTH

SEQ ID NO: 52 - protein, 6 aa, Artificial Sequence
  Amino acid sequence
GGLQGY

SEQ ID NO: 53 - protein, 6 aa, Artificial Sequence
  Amino acid sequence
GGLQGS

SEQ ID NO: 54 - protein, 15 aa, Artificial Sequence
  Amino acid sequence
AVDASRGLPYELYYY

SEQ ID NO: 55 - protein, 20 aa, Artificial Sequence
  Amino acid sequence
ALAVYGPNRYRYGPVGEYNY

SEQ ID NO: 56 - protein, 12 aa, Artificial Sequence
  Amino acid sequence
GYGATTTRPGRY

SEQ ID NO: 57 - protein, 18 aa, Artificial Sequence
  Amino acid sequence
DPSHYYSEYDCGYYGMDY

SEQ ID NO: 58 - protein, 12 aa, Artificial Sequence
  Amino acid sequence
DIGWPYVLDYDF

SEQ ID NO: 59 - protein, 17 aa, Artificial Sequence
  Amino acid sequence
DRRVYYDTYPNLRGYDY

SEQ ID NO: 60 - protein, 15 aa, Artificial Sequence
  Amino acid sequence
ARGPGSVGPSEEYNY

SEQ ID NO: 61 - protein, 18 aa, Artificial Sequence
  Amino acid sequence
ARGGGYRASGGPLSEYNY

SEQ ID NO: 62 - protein, 17 aa, Artificial Sequence
  Amino acid sequence
ALGSTGSGSTPVPEYRY

SEQ ID NO: 63 - protein, 17 aa, Artificial Sequence
  Amino acid sequence
ARGGVAGTDGPLGDYNY

SEQ ID NO: 64 - protein, 12 aa, Artificial Sequence
  Amino acid sequence
DIRYPTGLVGDY

SEQ ID NO: 65 - protein, 12 aa, Artificial Sequence
  Amino acid sequence
TTVMYDSNSPDY

SEQ ID NO: 66 - protein, 20 aa, Artificial Sequence
  Amino acid sequence
DPHILHNDRAGAFLVEDYDH

SEQ ID NO: 67 - protein, 25 aa, Artificial Sequence
  Amino acid sequence
EVQLVESGGGSVQAGGSLRLSCAAS

SEQ ID NO: 68 - protein, 25 aa, Artificial Sequence
  Amino acid sequence
KVQLVESGGGSVQAGGSLRLSCAAS

SEQ ID NO: 69 - protein, 25 aa, Artificial Sequence
  Amino acid sequence
EVQLVESGRGSVQAGGSLRLSCAAS

SEQ ID NO: 70 - protein, 25 aa, Artificial Sequence
  Amino acid sequence
EVQLVESGGGSVQTGGSLRLSCAAS

SEQ ID NO: 71 - protein, 25 aa, Artificial Sequence
  Amino acid sequence
EVQLVESEGGSVQAGGSLRLSCAAS

SEQ ID NO: 72 - protein, 25 aa, Artificial Sequence
  Amino acid sequence
EVQLVESRGGSVQAGGSLRLSCAAS

SEQ ID NO: 73 - protein, 25 aa, Artificial Sequence
  Amino acid sequence
DVQLVESGGGLVQPGGSLRLSCVAS

SEQ ID NO: 74 - protein, 25 aa, Artificial Sequence
  Amino acid sequence
DVQLVESGGGLVQPGGSLRLSCAAS

SEQ ID NO: 75 - protein, 25 aa, Artificial Sequence
  Amino acid sequence
EVQLVESGGALVRPGGSLRLSCAAS

SEQ ID NO: 76 - protein, 25 aa, Artificial Sequence [sequence omitted]

SEQ ID NO: 77 - protein, 25 aa, Artificial Sequence
  Amino acid sequence
DVQLVESGGGLVQPGGSLRLSCAGS

SEQ ID NO: 78 - protein, 25 aa, Artificial Sequence
  Amino acid sequence
EVQLVESGGGLVQPGGSLRLSCSAS

SEQ ID NO: 79 - protein, 25 aa, Artificial Sequence
  Amino acid sequence
EVQLVESEGGTVEPGESLRLACAAP

SEQ ID NO: 80 - protein, 14 aa, Artificial Sequence
  Amino acid sequence
WYRQAPGKQREFVA

SEQ ID NO: 81 - protein, 14 aa, Artificial Sequence
  Amino acid sequence
WYRQAPRKQREFVA

SEQ ID NO: 82 - protein, 14 aa, Artificial Sequence
  Amino acid sequence
WYRQAPGKQRELVA

SEQ ID NO: 83 - protein, 14 aa, Artificial Sequence
  Amino acid sequence
WFRQAPGKEREFVA

SEQ ID NO: 84 - protein, 14 aa, Artificial Sequence
  Amino acid sequence
WVRQAPGRGLEWVS

SEQ ID NO: 85 - protein, 14 aa, Artificial Sequence
  Amino acid sequence
WFRQAPGKEREGVS

SEQ ID NO: 86 - protein, 14 aa, Artificial Sequence
  Amino acid sequence
WHRQAPGKQRDLVA

SEQ ID NO: 87 - protein, 14 aa, Artificial Sequence
  Amino acid sequence
WYRQAPEKEREMVA

SEQ ID NO: 88 - protein, 39 aa, Artificial Sequence
  Amino acid sequence
YAVSVRGRFTISRDNAEGTGYLQMNSLKPEDTAVYYCNA

SEQ ID NO: 89 - protein, 39 aa, Artificial Sequence
  Amino acid sequence
YAVSVKGRFTISRDNAEGTGYLQMNSLKPEDTAVYYCNA

SEQ ID NO: 90 - protein, 39 aa, Artificial Sequence
  Amino acid sequence
YAVSVKGRFTISRDNAEGTGFLQMNGLKPEDTAVYYCNA

SEQ ID NO: 91 - protein, 39 aa, Artificial Sequence
  Amino acid sequence
YADSVKGRFTISRDNSKNTVYLQMNSLRPEDTAVYYCNA

SEQ ID NO: 92 - protein, 39 aa, Artificial Sequence
  Amino acid sequence
YADSVKGRFTISRDNSKNTVYLQMNSLRPEDTAVYYCTA

SEQ ID NO: 93 - protein, 39 aa, Artificial Sequence
  Amino acid sequence
YADSVKGRFTISRDNAKNTVYLQMNNLKPDDTAVYYCNT

SEQ ID NO: 94 - protein, 39 aa, Artificial Sequence
  Amino acid sequence
YADSVKGRFTISRDNAKNTMYLQMNNLKPEDTGVYYCAA

SEQ ID NO: 95 - protein, 39 aa, Artificial Sequence
  Amino acid sequence
YADSVKGRFTISRDNSKNTVYLQMNSLRPEDTAVYYCYA

SEQ ID NO: 96 - protein, 39 aa, Artificial Sequence
  Amino acid sequence
YADSVKGRFTISRDNSKNTVYLQMNSLRPEDTAVYYCAA

SEQ ID NO: 97 - protein, 39 aa, Artificial Sequence
  Amino acid sequence
YSDSVKGRFTISRDNSKNTVYLQMNSLRPEDTAVYYCTA

SEQ ID NO: 98 - protein, 39 aa, Artificial Sequence
  Amino acid sequence
YADSVKGRFTISRDNAENTVYLQMNDLKPEDTAVYYCHA

SEQ ID NO: 99 - protein, 39 aa, Artificial Sequence
  Amino acid sequence
YADSVKGRFTISSDNATSTFYLQMNSLQVEDTAVYYCAT

SEQ ID NO: 100 - protein, 11 aa, Artificial Sequence
  Amino acid sequence
WGLGTQVTVSS

SEQ ID NO: 101 - protein, 11 aa, Artificial Sequence
  Amino acid sequence
WGLGTLVTVSS

SEQ ID NO: 102 - protein, 11 aa, Artificial Sequence
  Amino acid sequence
WGQGTLVTVSS

SEQ ID NO: 103 - protein, 11 aa, Artificial Sequence
  Amino acid sequence
WGQGTQVTVSS

SEQ ID NO: 104 - protein, 11 aa, Artificial Sequence
  Amino acid sequence
WGKGTLVTVSS

SEQ ID NO: 105 - protein, 2415 aa, Artificial Sequence
  Amino acid sequence
MTTLLWVFVTLRVITAAVTVETSDHDNSLSVSIPQPSPLRVLLGTSLTIPCYFIDPMHPVTTAPSTAPLAPRIKWSRVSKEKEVVLLVATEGRVRVNSAYQDKVSLPNYPAIPSDATLEVQSLRSNDSGVYRCEVMHGIEDSEATLEVVVKGIVFHYRAISTRYTLDFDRAQRACLQNSAIIATPEQLQAAYEDGFHQCDAGWLADQTVRYPIHTPREGCYGDKDEFPGVRTYGIRDTNETYDVYCFAEEMEGEVFYATSPEKFTFQEAANECRRLGARLATTGHVYLAWQAGMDMCSAGWLADRSVRYPISKARPNCGGNLLGVRTVYVHANQTGYPDPSSRYDAICYTGEDFVDIPENFFGVGGEEDITVQTVTWPDMELPLPRNITEGEARGSVILTVKPIFEVSPSPLEPEEPFTFAPEIGATAFAEVENETGEATRPWGFPTPGLGPATAFTSEDLVVQVTAVPGQPHLPGGVVFHYRPGPTRYSLTFEEAQQACPGTGAVIASPEQLQAAYEAGYEQCDAGWLRDQTVRYPIVSPRTPCVGDKDSSPGVRTYGVRPSTETYDVYCFVDRLEGEVFFATRLEQFTFQEALEFCESHNATATTGQLYAAWSRGLDKCYAGWLADGSLRYPIVTPRPACGGDKPGVRTVYLYPNQTGLPDPLSRHHAFCFRGISAVPSPGEEEGGTPTSPSGVEEWIVTQVVPGVAAVPVEEETTAVPSGETTAILEFTTEPENQTEWEPAYTPVGTSPLPGILPTWPPTGAETEESTEGPSATEVPSASEEPSPSEVPFPSEEPSPSEEPFPSVRPFPSVELFPSEEPFPSKEPSPSEEPSASEEPYTPSPPEPSWTELPSSGEESGAPDVSGDFTGSGDVSGHLDFSGQLSGDRASGLPSGDLDSSGLTSTVGSGLTVESGLPSGDEERIEWPSTPTVGELPSGAEILEGSASGVGDLSGLPSGEVLETSASGVGDLSGLPSGEVLETTAPGVEDISGLPSGEVLETTAPGVEDISGLPSGEVLETTAPGVEDISGLPSGEVLETTAPGVEDISGLPSGEVLETTAPGVEDISGLPSGEVLETAAPGVEDISGLPSGEVLETAAPGVEDISGLPSGEVLETAAPGVEDISGLPSGEVLETAAPGVEDISGLPSGEVLETAAPGVEDISGLPSGEVLETAAPGVEDISGLPSGEVLETAAPGVEDISGLPSGEVLETAAPGVEDISGLPSGEVLETAAPGVEDISGLPSGEVLETAAPGVEDISGLPSGEVLETAAPGVEDISGLPSGEVLETTAPGVEEISGLPSGEVLETTAPGVDEISGLPSGEVLETTAPGVEEISGLPSGEVLETSTSAVGDLSGLPSGGEVLEISVSGVEDISGLPSGEVVETSASGIEDVSELPSGEGLETSASGVEDLSRLPSGEEVLEISASGFGDLSGVPSGGEGLETSASEVGTDLSGLPSGREGLETSASGAEDLSGLPSGKEDLVGSASGDLDLGKLPSGTLGSGQAPETSGLPSGFSGEYSGVDLGSGPPSGLPDFSGLPSGFPTVSLVDSTLVEVVTASTASELEGRGTIGISGAGEISGLPSSELDISGRASGLPSGTELSGQASGSPDVSGEIPGLFGVSGQPSGFPDTSGETSGVTELSGLSSGQPGVSGEASGVLYGTSQPFGITDLSGETSGVPDLSGQPSGLPGFSGATSGVPDLVSGTTSGSGESSGITFVDTSLVEVAPTTFKEEEGLGSVELSGLPSGEADLSGKSGMVDVSGQFSGTVDSSGFTSQTPEFSGLPSGIAEVSGESSRAEIGSSLPSGAYYGSGTPSSFPTVSLVDRTLVESVTQAPTAQEAGEGPSGILELSGAHSGAPDMSGEHSGFLDLSGLQSGLIEPSGEPPGTPYFSGDFASTTNVSGESSVAMGTSGEASGLPEVTLITSEFVEGVTEPTISQELGQRPPVTHTPQLFESSGKVSTAGDISGATPVLPGSGVEVSSVPESSSETSAYPEAGFGASAAPEASREDSGSPDLSETTSAFHEANLERSSGLGVSGSTLTFQEGEASAAPEVSGESTTTSDVGTEAPGLPSATPTASGDRTEISGDLSGHTSQLGVVISTSIPESEWTQQTQRPAETHLEIESSSLLYSGEETHTVETATSPTDASIPASPEWKRESESTAAAPARSCAEEPCGAGTCKETEGHVICLCPPGYTGEHCNIDQEVCEEGWNKYQGHCYRHFPDRETWVDAERRCREQQSHLSSIVTPEEQEFVNNNAQDYQWIGLNDRTIEGDFRWSDGHPMQFENWRPNQPDNFFAAGEDCVVMIWHEKGEWNDVPCNYHLPFTCKKGTVACGEPPVVEHARTFGQKKDRYEINSLVRYQCTEGFVQRHMPTIRCQPSGHWEEPRITCTDATTYKRRLQKRSSRHPRRSRPSTAH

SEQ ID NO: 106 - protein, 20 aa, Artificial Sequence
  Amino acid sequence
ALAVYGPSRYRYGPVGEYQY

SEQ ID NO: 107 - protein, 18 aa, Artificial Sequence
  Amino acid sequence
DPSHYYSEYECGYYGMDY

SEQ ID NO: 108 - protein, 14 aa, Artificial Sequence
  Amino acid sequence
WVRQAPGKGLEWVS

SEQ ID NO: 109 - protein, 123 aa, Artificial Sequence
  Amino acid sequence
EVQLVESGGGLVQPGGSLRLSCAASGSIFSINAMGWYRQAPGKQRELVAAISSGGSTYYADSVKGRFTISRDNSKNTVYLQMNSLRPEDTAVYYCNAAVDASRGLPYELYYYWGQGTLVTVSS

SEQ ID NO: 110 - protein, 129 aa, Artificial Sequence
  Amino acid sequence
DVQLVESGGGLVQPGGSLRLSCAASGRTFSSYAMGWFRQAPGKEREFVAAISWSGGSTYYADSVKGRFTISRDNSKNTVYLQMNSLRPEDTAVYYCTAALAVYGPSRYRYGPVGEYQYWGQGTLVTVSS

SEQ ID NO: 111 - protein, 121 aa, Artificial Sequence
  Amino acid sequence
EVQLVESGGGLVQPGGSLRLSCAASGFAFSAAYMSWVRQAPGKGLEWVSSISDDGSKTYYADSVKGRFTISRDNSKNTVYLQMNSLRPEDTAVYYCNTGYGATTTRPGRYWGQGTLVTVSS

SEQ ID NO: 112 - protein, 128 aa, Artificial Sequence
  Amino acid sequence
EVQLVESGGGLVQPGGSLRLSCAASGFTLAYYSIGWFRQAPGKEREGVSCISSGIDGSTYYADSVKGRFTISRDNSKNTLYLQMNSLRPEDTAVYYCAADPSHYYSEYECGYYGMDYWGQGTLVTVSS

SEQ ID NO: 113 - protein, 39 aa, Artificial Sequence
  Amino acid sequence
YADSVKGRFTISRDNSKNTVYLQMNSLRPEDTAVYYCNT

SEQ ID NO: 114 - protein, 39 aa, Artificial Sequence
  Amino acid sequence
YADSVKGRFTISRDNSKNTLYLQMNSLRPEDTAVYYCAA

SEQ ID NO: 115 - protein, 471 aa, Homo sapiens
  Amino acid sequence
MHPGVLAAFLFLSWTHCRALPLPSGGDEDDLSEEDLQFAERYLRSYYHPTNLAGILKENAASSMTERLREMQSFFGLEVTGKLDDNTLDVMKKPRCGVPDVGEYNVFPRTLKWSKMNLTYRIVNYTPDMTHSEVEKAFKKAFKVWSDVTPLNFTRLHDGIADIMISFGIKEHGDFYPFDGPSGLLAHAFPPGPNYGGDAHFDDDETWTSSSKGYNLFLVAAHEFGHSLGLDHSKDPGALMFPIYTYTGKSHFMLPDDDVQGIQSLYGPGDEDPNPKHPKTPDKCDPSLSLDAITSLRGETMIFKDRFFWRLHPQQVDAELFLTKSFWPELPNRIDAAYEHPSHDLIFIFRGRKFWALNGYDILEGYPKKISELGLPKEVKKISAAVHFEDTGKTLLFSGNQVWRYDDTNHIMDKDYPRLIEEDFPGIGDKVDAVYEKNGYIYFFNGPIQFEYSIWSNRIVRVMPANSILWC

SEQ ID NO: 116 - protein, 471 aa, Pan troglodytes
  Amino acid sequence
MHPGVLAAFLFLSWAHCRALPLPSGGDEDDLSEEDLQFAERYLRSYYHPTNLAGILKENAASSMTERLREMQSFFGLEVTGKLDDNTLDVMKKPRCGVPDVGEYNVFPRTLKWSKMNLTYRIVNYTPDMTHSEVEKAFKKAFKVWSDVTPLNFTRLHDGIADIMISFGIKEHGDFYPFDGPSGLLAHAFPPGPNYGGDAHFDDDETWTSSSKGYNLFLVAAHEFGHSLGLDHSKDPGALMFPIYTYTGKSHFMLPDDDVQGIQSLYGPGDEDPNPKHPKTPDKCDPSLSLDAITSLRGETMIFKDRFFWRLHPQQVDAELFLTKSFWPELPNRIDAAYEHPSHDLIFIFRGRKFWALNGYDILEGYPKKISELGLPKEVKKISATVHFEDTGKTLLFSGNQVWRYDDTNHIMDKDYPRLIEEEFPGIGDKVDAVYEKNGYIYFFNGPIQFEYSIWSNRIVRVMPANSILWC

SEQ ID NO: 117 - protein, 471 aa, Macaca mulatta
  Amino acid sequence
MHPGVLAAFLFLSWTHCRALPLPSGGDEDDLSEEDLQFAERYLRSYYYPTNLAGILKENAASSMTDRLREMQSFFGLEVTGKLDDNTLDVMKKPRCGVPDVGEYNVFPRTLKWSKMNLTYRIVNYTPDMTHSEVEKAFKKAFKVWSDVTPLNFTRLHDGIADIMISFGTKEHGDFYPFDGPSGLLAHAFPPGPNYGGDAHFDDDETWTSSSKGYNLFLVAAHEFGHSLGLDHSKDPGALMFPIYTYTGKSHFMLPDDDVQGIQSLYGPGDEDPNPKHPKTPDKCDPSLSLDAITSLRGETMIFKDRFFWRLHPQQVDAELFLTKSFWPELPNRIDAAYEHPSHDLIFIFRGRKFWALNGYDILEGYPKKISELGFPKEVKKISAAVHFEDTGKTLLFSGNQVWRYDDTNHIMDKDYPRLIEEDFPGIGDKVDAVYEKNGYIYFFNGPIQFEYSIWSNRIVRVMPANSILWC

SEQ ID NO: 118 - protein, 496 aa, Canis lupus
  Amino acid sequence
MSHHCRSIKVKVLVWERQQAPGTTTKMLPGILAAFLCLSWTQCWSLPLPSDGDDDLSEEDFQLAERYLKSYYYPLNPAGILKKSAAGSVADRLREMQSFFGLEVTGKLDDNTLDIMKKPRCGVPDVGEYNVFPRTLKWSKTNLTYRIVNYTPDLTHSEVEKAFKKAFKVWSDVTPLNFTRLHDGTADIMISFGTKEHGDFYPFDGPSGLLAHAFPPGPNYGGDAHFDDDETWTSSSKGYNLFLVAAHEFGHSLGLDHSKDPGALMFPIYTYTGKSHFMLPDDDVQGIQSLYGPGDEDPNPRHPKTPDKCDPSLSLDAITSLRGETMIFKDRFFWRLHPQQVDAELFLTKSFWPELPNRIDAAYEHPSRDLIFIFRGRKYWALNGYDILEGYPQKISELGFPKEVKKISAAVHFEDTGKTLFFSGNQVWSYDDTNQIMDKDYPRLIEEDFPGIGDKVDAVYEKNGYIYFFNGPIQFEYNIWSKRIVRVMPANSLLWC

SEQ ID NO: 119 - protein, 471 aa, Bos taurus
  Amino acid sequence
MHPRVLAGFLFFSWTACWSLPLPSDGDSEDLSEEDFQFAESYLKSYYYPQNPAGILKKTAASSVIDRLREMQSFFGLEVTGRLDDNTLDIMKKPRCGVPDVGEYNVFPRTLKWSKMNLTYRIVNYTPDLTHSEVEKAFRKAFKVWSDVTPLNFTRIHNGTADIMISFGTKEHGDFYPFDGPSGLLAHAFPPGPNYGGDAHFDDDETWTSSSKGYNLFLVAAHEFGHSLGLDHSKDPGALMFPIYTYTGKSHFMLPDDDVQGIQSLYGPGDEDPYSKHPKTPDKCDPSLSLDAITSLRGETLIFKDRFFWRLHPQQVEAELFLTKSFGPELPNRIDAAYEHPSHDLIFIFRGRKFWALSGYDILEDYPKKISELGFPKHVKKISAALHFEDSGKTLFFSENQVWSYDDTNHVMDKDYPRLIEEVFPGIGDKVDAVYQKNGYIYFFNGPIQFEYSIWSNRIVRVMTTNSLLWC

SEQ ID NO: 120 - protein, 472 aa, Mus musculus
  Amino acid sequence
MHSAILATFFLLSWTPCWSLPLPYGDDDDDDLSEEDLVFAEHYLKSYYHPATLAGILKKSTVTSTVDRLREMQSFFGLEVTGKLDDPTLDIMRKPRCGVPDVGEYNVFPRTLKWSQTNLTYRIVNYTPDMSHSEVEKAFRKAFKVWSDVTPLNFTRIYDGTADIMISFGTKEHGDFYPFDGPSGLLAHAFPPGPNYGGDAHFDDDETWTSSSKGYNLFIVAAHELGHSLGLDHSKDPGALMFPIYTYTGKSHFMLPDDDVQGIQFLYGPGDEDPNPKHPKTPEKCDPALSLDAITSLRGETMIFKDRFFWRLHPQQVEAELFLTKSFWPELPNHVDAAYEHPSRDLMFIFRGRKFWALNGYDILEGYPRKISDLGFPKEVKRLSAAVHFENTGKTLFFSENHVWSYDDVNQTMDKDYPRLIEEEFPGIGNKVDAVYEKNGYIYFFNGPIQFEYSIWSNRIVRVMPTNSILWC

SEQ ID NO: 121 - protein, 472 aa, Rattus norvegicus
  Amino acid sequence
MHSAILATFFLLSWTHCWSLPLPYGDDDDDDLSEEDLEFAEHYLKSYYHPVTLAGILKKSTVTSTVDRLREMQSFFGLDVTGKLDDPTLDIMRKPRCGVPDVGEYNVFPRTLKWSQTNLTYRIVNYTPDISHSEVEKAFRKAFKVWSDVTPLNFTRIHDGTADIMISFGTKEHGDFYPFDGPSGLLAHAFPPGPNLGGDAHFDDDETWTSSSKGYNLFIVAAHELGHSLGLDHSKDPGALMFPIYTYTGKSHFMLPDDDVQGIQSLYGPGDEDPNPKHPKTPEKCDPALSLDAITSLRGETMIFKDRFFWRLHPQQVEPELFLTKSFWPELPNHVDAAYEHPSRDLMFIFRGRKFWALNGYDIMEGYPRKISDLGFPKEVKRLSAAVHFEDTGKTLFFSGNHVWSYDDANQTMDKDYPRLIEEEFPGIGDKVDAVYEKNGYIYFFNGPIQFEYSIWSNRIVRVMPTNSLLWC

SEQ ID NO: 122 - protein, 471 aa, Gallus gallus
  Amino acid sequence
MQPRLSAVFFFLLGLSFCLTVPIPLDDSHEFTEEDLRFAERYLRTHYDLRPNPTGIMKKSANTMASKLREMQAFFGLEVTGKLDEETYELMQKPRCGVPDVGEYNFFPRKLKWSNTNLTYRIMSYTSDLRRAEVERAFKRAFKVWSDVTPLNFTRIRSGTADIMISFGTKEHGDFYPFDGPSGLLAHAFPPGPDYGGDAHFDDDETWSDDSRGYNLFLVAAHEFGHSLGLEHSRDPGALMFPIYTYTGKSGFVLPDDDVQGIQELYGAGDRDPNPKHPKTPEKCAADLSIDAITKLRGEMLVFKDRFFWRLHPQMVEAELVLIKSFWPELPNKIDAAYENPIKDLVFMFKGKKVWAMNGYDIVEGFPKKIYEMGFPKEMKRIDAVVHIDDTGKTLFFTGNKYWSYDEETEVMDTGYPKFIEDEFAGIGDRVDAVYHRNGYLYFFNGPLQFEYSIWSKRIVRILHTNSLFWC

SEQ ID NO: 123 - protein, 23 aa, Artificial Sequence
  Amino acid sequence
AAAEQKLISEEDLNGAAHHHHHH

SEQ ID NO: 124 - protein, 34 aa, Artificial Sequence
  Amino acid sequence
AAADYKDHDGDYKDHDIDYKDDDDKGAAHHHHHH

SEQ ID NO: 125 - skipped

SEQ ID NO: 126 - protein, 5 aa, Artificial Sequence
  Amino acid sequence
GGGGS

SEQ ID NO: 127 - protein, 7 aa, Artificial Sequence
  Amino acid sequence
SGGSGGS

SEQ ID NO: 128 - protein, 8 aa, Artificial Sequence
  Amino acid sequence
GGGGGGGS

SEQ ID NO: 129 - protein, 9 aa, Artificial Sequence
  Amino acid sequence
GGGGSGGGS

SEQ ID NO: 130 - protein, 10 aa, Artificial Sequence
  Amino acid sequence
GGGGSGGGGS

SEQ ID NO: 131 - protein, 15 aa, Artificial Sequence
  Amino acid sequence
GGGGSGGGGSGGGGS

SEQ ID NO: 132 - protein, 18 aa, Artificial Sequence
  Amino acid sequence
GGGGSGGGGSGGGGGGGS

SEQ ID NO: 133 - protein, 20 aa, Artificial Sequence
  Amino acid sequence
GGGGSGGGGSGGGGSGGGGS

SEQ ID NO: 134 - protein, 25 aa, Artificial Sequence
  Amino acid sequence
GGGGSGGGGSGGGGSGGGGSGGGGS

SEQ ID NO: 135 - protein, 30 aa, Artificial Sequence
  Amino acid sequence
GGGGSGGGGSGGGGSGGGGSGGGGSGGGGS

SEQ ID NO: 136 - protein, 35 aa, Artificial Sequence
  Amino acid sequence
GGGGSGGGGSGGGGSGGGGSGGGGSGGGGSGGGGS

SEQ ID NO: 137 - protein, 40 aa, Artificial Sequence
  Amino acid sequence
GGGGSGGGGSGGGGSGGGGSGGGGSGGGGSGGGGSGGGGS

SEQ ID NO: 138 - protein, 15 aa, Artificial Sequence
  Amino acid sequence
EPKSCDKTHTCPPCP

SEQ ID NO: 139 - protein, 24 aa, Artificial Sequence
  Amino acid sequence
GGGGSGGGSEPKSCDKTHTCPPCP

SEQ ID NO: 140 - protein, 12 aa, Artificial Sequence
  Amino acid sequence
EPKTPKPQPAAA

SEQ ID NO: 141 - protein, 62 aa, Artificial Sequence
  Amino acid sequence
ELKTPLGDTTHTCPRCPEPKSCDTPPPCPRCPEPKSCDTPPPCPRCPEPKSCDTPPPCPRCP

SEQ ID NO: 142 - protein, 115 aa, Artificial Sequence [sequence omitted]

SEQ ID NO: 143 - protein, 115 aa, Artificial Sequence [sequence omitted]

SEQ ID NO: 144 - protein, 116 aa, Artificial Sequence
  Amino acid sequence
EVQLVESGGGVVQPGNSLRLSCAASGFTFSSFGMSWVRQAPGKGLEWVSSISGSGSDTLYADSVKGRFTISRDNAKTTLYLQMNSLRPEDTATYYCTIGGSLSRSSQGTLVTVSSA

SEQ ID NO: 145 - protein, 116 aa, Artificial Sequence
  Amino acid sequence
EVQLVESGGGVVQPGGSLRLSCAASGFTFRSFGMSWVRQAPGKGPEWVSSISGSGSDTLYADSVKGRFTISRDNSKNTLYLQMNSLRPEDTATYYCTIGGSLSRSSQGTLVTVSSA

SEQ ID NO: 146 - protein, 115 aa, Artificial Sequence [sequence omitted]

SEQ ID NO: 147 - protein, 116 aa, Artificial Sequence
  Amino acid sequence
EVQLVESGGGLVQPGNSLRLSCAASGFTFSSFGMSWVRQAPGKGLEWVSSISGSGSDTLYADSVKGRFTISRDNAKTTLYLQMNSLRPEDTAVYYCTIGGSLSRSSQGTLVKVSSA

SEQ ID NO: 148 - protein, 115 aa, Artificial Sequence
  Amino acid sequence
EVQLVESGGGVVQPGNSLRLSCAASGFTFSSFGMSWVRQAPGKGLEWVSSISGSGSDTLYADSVKGRFTISRDNAKTTLYLQMNSLRPEDTALYYCTIGGSLSRSSQGTLVTVSS

SEQ ID NO: 149 - protein, 116 aa, Artificial Sequence
  Amino acid sequence
EVQLVESGGGVVQPGNSLRLSCAASGFTFSSFGMSWVRQAPGKGLEWVSSISGSGSDTLYADSVKGRFTISRDNAKTTLYLQMNSLRPEDTALYYCTIGGSLSRSSQGTLVTVSSA

SEQ ID NO: 150 - protein, 117 aa, Artificial Sequence
  Amino acid sequence
EVQLVESGGGVVQPGNSLRLSCAASGFTFSSFGMSWVRQAPGKGLEWVSSISGSGSDTLYADSVKGRFTISRDNAKTTLYLQMNSLRPEDTALYYCTIGGSLSRSSQGTLVTVSSAA

SEQ ID NO: 151 - protein, 118 aa, Artificial Sequence
  Amino acid sequence
EVQLVESGGGVVQPGNSLRLSCAASGFTFSSFGMSWVRQAPGKGLEWVSSISGSGSDTLYADSVKGRFTISRDNAKTTLYLQMNSLRPEDTALYYCTIGGSLSRSSQGTLVTVSSAAA

SEQ ID NO: 152 - protein, 116 aa, Artificial Sequence
  Amino acid sequence
EVQLVESGGGVVQPGNSLRLSCAASGFTFSSFGMSWVRQAPGKGLEWVSSISGSGSDTLYADSVKGRFTISRDNAKTTLYLQMNSLRPEDTALYYCTIGGSLSRSSQGTLVTVSSG

SEQ ID NO: 153 - protein, 117 aa, Artificial Sequence
  Amino acid sequence
EVQLVESGGGVVQPGNSLRLSCAASGFTFSSFGMSWVRQAPGKGLEWVSSISGSGSDTLYADSVKGRFTISRDNAKTTLYLQMNSLRPEDTALYYCTIGGSLSRSSQGTLVTVSSGG

SEQ ID NO: 154 - protein, 118 aa, Artificial Sequence
  Amino acid sequence
EVQLVESGGGVVQPGNSLRLSCAASGFTFSSFGMSWVRQAPGKGLEWVSSISGSGSDTLYADSVKGRFTISRDNAKTTLYLQMNSLRPEDTALYYCTIGGSLSRSSQGTLVTVSSGGG

SEQ ID NO: 155 - protein, 115 aa, Artificial Sequence
  Amino acid sequence
EVQLVESGGGVVQPGGSLRLSCAASGFTFRSFGMSWVRQAPGKGPEWVSSISGSGSDTLYADSVKGRFTISRDNSKNTLYLQMNSLRPEDTALYYCTIGGSLSRSSQGTLVTVSS

SEQ ID NO: 156 - protein, 116 aa, Artificial Sequence
  Amino acid sequence
EVQLVESGGGVVQPGGSLRLSCAASGFTFRSFGMSWVRQAPGKGPEWVSSISGSGSDTLYADSVKGRFTISRDNSKNTLYLQMNSLRPEDTALYYCTIGGSLSRSSQGTLVTVSSA

SEQ ID NO: 157 - protein, 5 aa, Artificial Sequence
  Amino acid sequence
SFGMS

SEQ ID NO: 158 - protein, 17 aa, Artificial Sequence
  Amino acid sequence
SISGSGSDTLYADSVKG

SEQ ID NO: 159 - protein, 6 aa, Artificial Sequence
  Amino acid sequence
GGSLSR

SEQ ID NO: 160 - protein, 278 aa, Artificial Sequence
  Amino acid sequence
EVQLVESGGGLVQPGGSLRLSCAASGRTFSSYAMGWFRQAPGKEREFVAAISWSGGSTYYADSVKGRFTISRDNSKNTVYLQMNSLRPEDTAVYYCTAALAVYGPNRYRYGPVGEYNYWGQGTLVTVSSGGGGSGGGGSGGGGSGGGGSGGGGSGGGGSGGGGSEVQLVESGGGSVQAGGSLRLSCAASGSTFSRYSMNWYRQAPGKQREFVAGISVGRITNYAVSVRGRFTISRDNAEGTGYLQMNSLKPEDTAVYYCNAGGLQGYWGLGTLVTVSS

SEQ ID NO: 161 - protein, 269 aa, Artificial Sequence
  Amino acid sequence
EVQLVESGGGLVQPGGSLRLSCAGSGSIFRINVMAWYRQAPGKQRELVAAITSGGTTNYADSVKGRFTISRDNSKNTVYLQMNSLRPEDTAVYYCYADIGWPYVLDYDFWGQGTLVTVSSGGGGSGGGGSGGGGSGGGGSGGGGSGGGGSGGGGSEVQLVESGGGSVQAGGSLRLSCAASGSTFSRYSMNWYRQAPGKQREFVAGISVGRITNYAVSVRGRFTISRDNAEGTGYLQMNSLKPEDTAVYYCNAGGLQGYWGLGTLVTVSS

SEQ ID NO: 162 - protein, 270 aa, Artificial Sequence
  Amino acid sequence
EVQLVESGGALVRPGGSLRLSCAASGFAFSAAYMSWVRQAPGRGLEWVSSISDDGSKTYYADSVKGRFTISRDNAKNTVYLQMNNLKPDDTAVYYCNTGYGATTTRPGRYWGQGTLVTVSSGGGGSGGGGSGGGGSGGGGSGGGGSGGGGSGGGGSEVQLVESGGGSVQAGGSLRLSCAASGSTFSRYSMNWYRQAPGKQREFVAGISVGRITNYAVSVRGRFTISRDNAEGTGYLQMNSLKPEDTAVYYCNAGGLQGYWGLGTLVTVSS

SEQ ID NO: 163 - protein, 278 aa, Artificial Sequence
  Amino acid sequence
EVQLVESGGGSVQAGGSLRLSCAASGSTFSRYSMNWYRQAPGKQREFVAGISVGRITNYAVSVRGRFTISRDNAEGTGYLQMNSLKPEDTAVYYCNAGGLQGYWGLGTLVTVSSGGGGSGGGGSGGGGSGGGGSGGGGSGGGGSGGGGSEVQLVESGGGLVQPGGSLRLSCAASGRTFSSYAMGWFRQAPGKEREFVAAISWSGGSTYYADSVKGRFTISRDNSKNTVYLQMNSLRPEDTAVYYCTAALAVYGPNRYRYGPVGEYNYWGQGTLVTVSS

SEQ ID NO: 164 - protein, 269 aa, Artificial Sequence
  Amino acid sequence
EVQLVESGGGSVQAGGSLRLSCAASGSTFSRYSMNWYRQAPGKQREFVAGISVGRITNYAVSVRGRFTISRDNAEGTGYLQMNSLKPEDTAVYYCNAGGLQGYWGLGTLVTVSSGGGGSGGGGSGGGGSGGGGSGGGGSGGGGSGGGGSEVQLVESGGGLVQPGGSLRLSCAGSGSIFRINVMAWYRQAPGKQRELVAAITSGGTTNYADSVKGRFTISRDNSKNTVYLQMNSLRPEDTAVYYCYADIGWPYVLDYDFWGQGTLVTVSS

SEQ ID NO: 165 - protein, 270 aa, Artificial Sequence
  Amino acid sequence
EVQLVESGGGSVQAGGSLRLSCAASGSTFSRYSMNWYRQAPGKQREFVAGISVGRITNYAVSVRGRFTISRDNAEGTGYLQMNSLKPEDTAVYYCNAGGLQGYWGLGTLVTVSSGGGGSGGGGSGGGGSGGGGSGGGGSGGGGSGGGGSEVQLVESGGALVRPGGSLRLSCAASGFAFSAAYMSWVRQAPGRGLEWVSSISDDGSKTYYADSVKGRFTISRDNAKNTVYLQMNNLKPDDTAVYYCNTGYGATTTRPGRYWGQGTLVTVSS

SEQ ID NO: 166 - protein, 121 aa, Artificial Sequence
  Amino acid sequence
EVQLVESGGGLVQPGGSLRLSCAASGSTFIINVVRWYRRAPGKQRELVATISSGGNANYVDSVRGRFTISRDNSKNTVYLQMNSLRPEDTAVYYCNVPTTHYGGVYYGPYWGQGTLVTVSS

SEQ ID NO: 167 - protein, 122 aa, Artificial Sequence
  Amino acid sequence
EVQLVESGGGVVQPGGSLRLSCAASGSTFIINVVRWYRRAPGKQRELVATISSGGNANYVDSVRGRFTISRDNSKNTVYLQMNSLRPEDTALYYCNVPTTHYGGVYYGPYWGQGTLVTVSSA

SEQ ID NO: 168 - protein, 125 aa, Artificial Sequence
  Amino acid sequence
EVQLVESGGGVVQPGGSLRLSCAASGRTFSSYTMGWFRQAPGKEREFVAAISWSGGRTYYADSVKGRFTISRDNSKNTVYLQMNSLRPEDTALYYCAAYRRRRASSNRGLWDYWGQGTLVTVSSA

SEQ ID NO: 169 - protein, 10 aa, Artificial Sequence
  Amino acid sequence
GSTFIINVVR

SEQ ID NO: 170 - protein, 9 aa, Artificial Sequence
  Amino acid sequence
TISSGGNAN

SEQ ID NO: 171 - protein, 13 aa, Artificial Sequence
  Amino acid sequence
PTTHYGGVYYGPY

SEQ ID NO: 172 - protein, 10 aa, Artificial Sequence
  Amino acid sequence
GRTFSSYTMG

SEQ ID NO: 173 - protein, 10 aa, Artificial Sequence
  Amino acid sequence
AISWSGGRTY

SEQ ID NO: 174 - protein, 15 aa, Artificial Sequence
  Amino acid sequence
YRRRRASSNRGLWDY

SEQ ID NO: 175 - protein, 17 aa, Artificial Sequence
  Amino acid sequence
AAAEQKLISEEDLNGAA

SEQ ID NO: 176 - protein, 277 aa, Artificial Sequence
  Amino acid sequence
EVQLVESGGGLVQPGGSLRLSCAASGFAFSAAYMSWVRQAPGKGLEWVSSISDDGSKTYYADSVKGRFTISRDNSKNTVYLQMNSLRPEDTAVYYCNTGYGATTTRPGRYWGQGTLVTVSSGGGGSGGGGSGGGGSGGGGSGGGGSGGGGSGGGGSEVQLVESGGGLVQPGGSLRLSCAASGSTFIINVVRWYRRAPGKQRELVATISSGGNANYVDSVRGRFTISRDNSKNTVYLQMNSLRPEDTAVYYCNVPTTHYGGVYYGPYWGQGTLVTVSS

SEQ ID NO: 177 - protein, 433 aa, Artificial Sequence
  Amino acid sequence
EVQLVESGGGLVQPGGSLRLSCAASGFAFSAAYMSWVRQAPGKGLEWVSSISDDGSKTYYADSVKGRFTISRDNSKNTVYLQMNSLRPEDTAVYYCNTGYGATTTRPGRYWGQGTLVTVSSGGGGSGGGGSGGGGSGGGGSGGGGSGGGGSGGGGSEVQLVESGGGLVQPGGSLRLSCAASGSTFIINVVRWYRRAPGKQRELVATISSGGNANYVDSVRGRFTISRDNSKNTVYLQMNSLRPEDTAVYYCNVPTTHYGGVYYGPYWGQGTLVTVSSGGGGSGGGGSGGGGSGGGGSGGGGSGGGGSGGGGSEVQLVESGGGLVQPGGSLRLSCAASGSTFIINVVRWYRRAPGKQRELVATISSGGNANYVDSVRGRFTISRDNSKNTVYLQMNSLRPEDTAVYYCNVPTTHYGGVYYGPYWGQGTLVTVSS

SEQ ID NO: 178 - protein, 280 aa, Artificial Sequence
  Amino acid sequence
EVQLVESGGGLVQPGGSLRLSCAASGFAFSAAYMSWVRQAPGKGLEWVSSISDDGSKTYYADSVKGRFTISRDNSKNTVYLQMNSLRPEDTAVYYCNTGYGATTTRPGRYWGQGTLVTVSSGGGGSGGGGSGGGGSGGGGSGGGGSGGGGSGGGGSEVQLVESGGGLVQPGGSLRLSCAASGRTFSSYTMGWFRQAPGKEREFVAAISWSGGRTYYADSVKGRFTISRDNSKNTVYLQMNSLRPEDTAVYYCAAYRRRRASSNRGLWDYWGQGTLVTVSS

SEQ ID NO: 179 - protein, 284 aa, Artificial Sequence
  Amino acid sequence
EVQLVESGGGLVQPGGSLRLSCAASGFTLAYYSIGWFRQAPGKEREGVSCISSGIDGSTYYADSVKGRFTISRDNAKNTMYLQMNNLKPEDTGVYYCAADPSHYYSEYDCGYYGMDYWGKGTLVTVSSGGGGSGGGGSGGGGSGGGGSGGGGSGGGGSGGGGSEVQLVESGGGLVQPGGSLRLSCAASGSTFIINVVRWYRRAPGKQRELVATISSGGNANYVDSVRGRFTISRDNSKNTVYLQMNSLRPEDTAVYYCNVPTTHYGGVYYGPYWGQGTLVTVSS

SEQ ID NO: 180 - protein, 440 aa, Artificial Sequence
  Amino acid sequence
EVQLVESGGGLVQPGGSLRLSCAASGFTLAYYSIGWFRQAPGKEREGVSCISSGIDGSTYYADSVKGRFTISRDNAKNTMYLQMNNLKPEDTGVYYCAADPSHYYSEYDCGYYGMDYWGKGTLVTVSSGGGGSGGGGSGGGGSGGGGSGGGGSGGGGSGGGGSEVQLVESGGGLVQPGGSLRLSCAASGSTFIINVVRWYRRAPGKQRELVATISSGGNANYVDSVRGRFTISRDNSKNTVYLQMNSLRPEDTAVYYCNVPTTHYGGVYYGPYWGQGTLVTVSSGGGGSGGGGSGGGGSGGGGSGGGGSGGGGSGGGGSEVQLVESGGGLVQPGGSLRLSCAASGSTFIINVVRWYRRAPGKQRELVATISSGGNANYVDSVRGRFTISRDNSKNTVYLQMNSLRPEDTAVYYCNVPTTHYGGVYYGPYWGQGTLVTVSS

SEQ ID NO: 181 - protein, 287 aa, Artificial Sequence
  Amino acid sequence
EVQLVESGGGLVQPGGSLRLSCAASGFTLAYYSIGWFRQAPGKEREGVSCISSGIDGSTYYADSVKGRFTISRDNAKNTMYLQMNNLKPEDTGVYYCAADPSHYYSEYDCGYYGMDYWGKGTLVTVSSGGGGSGGGGSGGGGSGGGGSGGGGSGGGGSGGGGSEVQLVESGGGLVQPGGSLRLSCAASGRTFSSYTMGWFRQAPGKEREFVAAISWSGGRTYYADSVKGRFTISRDNSKNTVYLQMNSLRPEDTAVYYCAAYRRRRASSNRGLWDYWGQGTLVTVSS

SEQ ID NO: 182 - protein, 438 aa, Artificial Sequence
  Amino acid sequence
DVQLVESGGGLVQPGGSLRLSCAASGRTFSSYAMGWFRQAPGKEREFVAAISWSGGSTYYADSVKGRFTISRDNSKNTVYLQMNSLRPEDTAVYYCTAALAVYGPSRYRYGPVGEYQYWGQGTLVTVSSGGGGSGGGGSGGGGSGGGGSGGGGSGGGGSGGGGSEVQLVESGGGLVQPGGSLRLSCAASGSTFSRYSMNWYRQAPGKQREFVAGISVGRITNYAVSVKGRFTISRDNSKNTGYLQMNSLRPEDTAVYYCNAGGLQGYWGQGTLVTVSSGGGGSGGGGSGGGGSGGGGSGGGGSGGGGSGGGGSEVQLVESGGGLVQPGGSLRLSCAASGRTFSSYTMGWFRQAPGKEREFVAAISWSGGRTYYADSVKGRFTISRDNSKNTVYLQMNSLRPEDTAVYYCAAYRRRRASSNRGLWDYWGQGTLVTVSSA

SEQ ID NO: 183 - protein, 434 aa, Artificial Sequence
  Amino acid sequence
EVQLVESGGGLVQPGGSLRLSCAASGRTFSSYAMGWFRQAPGKEREFVAAISWSGGSTYYADSVKGRFTISRDNSKNTVYLQMNSLRPEDTAVYYCTAALAVYGPSRYRYGPVGEYQYWGQGTLVTVSSGGGGSGGGGSGGGGSGGGGSGGGGSGGGGSGGGGSEVQLVESGGGSVQPGGSLRLSCAASGSTFSRYSMNWYRQAPGKQREFVAGISVGRITNYAVSVRGRFTISRDNSEGTGYLQMNSLRPEDTAVYYCNAGGLQGYWGLGTLVTVSSGGGGSGGGGSGGGGSGGGGSGGGGSGGGGSGGGGSEVQLVESGGGLVQPGGSLRLSCAASGSTFIINVVRWYRRAPGKQRELVATISSGGNANYVDSVRGRFTISRDNSKNTVYLQMNSLRPEDTAVYYCNVPTTHYGGVYYGPYWGQGTLVTVSS

SEQ ID NO: 184 - protein, 590 aa, Artificial Sequence
  Amino acid sequence
EVQLVESGGGLVQPGGSLRLSCAASGRTFSSYAMGWFRQAPGKEREFVAAISWSGGSTYYADSVKGRFTISRDNSKNTVYLQMNSLRPEDTAVYYCTAALAVYGPSRYRYGPVGEYQYWGQGTLVTVSSGGGGSGGGGSGGGGSGGGGSGGGGSGGGGSGGGGSEVQLVESGGGSVQPGGSLRLSCAASGSTFSRYSMNWYRQAPGKQREFVAGISVGRITNYAVSVRGRFTISRDNSEGTGYLQMNSLRPEDTAVYYCNAGGLQGYWGLGTLVTVSSGGGGSGGGGSGGGGSGGGGSGGGGSGGGGSGGGGSEVQLVESGGGLVQPGGSLRLSCAASGSTFIINVVRWYRRAPGKQRELVATISSGGNANYVDSVRGRFTISRDNSKNTVYLQMNSLRPEDTAVYYCNVPTTHYGGVYYGPYWGQGTLVTVSSGGGGSGGGGSGGGGSGGGGSGGGGSGGGGSGGGGSEVQLVESGGGLVQPGGSLRLSCAASGSTFIINVVRWYRRAPGKQRELVATISSGGNANYVDSVRGRFTISRDNSKNTVYLQMNSLRPEDTAVYYCNVPTTHYGGVYYGPYWGQGTLVTVSS

SEQ ID NO: 185 - protein, 437 aa, Artificial Sequence
  Amino acid sequence
EVQLVESGGGLVQPGGSLRLSCAASGRTFSSYAMGWFRQAPGKEREFVAAISWSGGSTYYADSVKGRFTISRDNSKNTVYLQMNSLRPEDTAVYYCTAALAVYGPSRYRYGPVGEYQYWGQGTLVTVSSGGGGSGGGGSGGGGSGGGGSGGGGSGGGGSGGGGSEVQLVESGGGSVQPGGSLRLSCAASGSTFSRYSMNWYRQAPGKQREFVAGISVGRITNYAVSVRGRFTISRDNSEGTGYLQMNSLRPEDTAVYYCNAGGLQGYWGLGTLVTVSSGGGGSGGGGSGGGGSGGGGSGGGGSGGGGSGGGGSEVQLVESGGGLVQPGGSLRLSCAASGRTFSSYTMGWFRQAPGKEREFVAAISWSGGRTYYADSVKGRFTISRDNSKNTVYLQMNSLRPEDTAVYYCAAYRRRRASSNRGLWDYWGQGTLVTVSS

SEQ ID NO: 186 - protein, 278 aa, Artificial Sequence
  Amino acid sequence
EVQLVESGGGLVQPGGSLRLSCAASGRTFSSYAMGWFRQAPGKEREFVAAISWSGGSTYYADSVKGRFTISRDNSKNTVYLQMNSLRPEDTAVYYCTAALAVYGPSRYRYGPVGEYQYWGQGTLVTVSSGGGGSGGGGSGGGGSGGGGSGGGGSGGGGSGGGGSEVQLVESGGGLVQPGGSLRLSCAASGSTFSRYSMNWYRQAPGKQREFVAGISVGRITNYAVSVKGRFTISRDNSKNTVYLQMNSLRPEDTAVYYCNAGGLQGYWGQGTLVTVSS

SEQ ID NO: 187 - protein, 278 aa, Artificial Sequence
  Amino acid sequence
EVQLVESGGGLVQPGGSLRLSCAASGRTFSSYAMGWFRQAPGKEREFVAAISWSGGSTYYADSVKGRFTISRDNSKNTVYLQMNSLRPEDTAVYYCTAALAVYGPSRYRYGPVGEYQYWGQGTLVTVSSGGGGSGGGGSGGGGSGGGGSGGGGSGGGGSGGGGSEVQLVESGGGLVQPGGSLRLSCAASGSTFSRYSMNWYRQAPGKQREFVAGISVGRITNYAVSVKGRFTISRDNSKNTGYLQMNSLRPEDTAVYYCNAGGLQGYWGQGTLVTVSS

SEQ ID NO: 188 - protein, 283 aa, Artificial Sequence
  Amino acid sequence
DVQLVESGGGLVQPGGSLRLSCAASGSIFSINAMGWYRQAPGKQRELVAAISSGGSTYYADSVKGRFTISRDNSKNTVYLQMNSLRPEDTAVYYCNAAVDASRGLPYELYYYWGQGTLVTVSSGGGGSGGGGSGGGGSGGGGSGGGGSGGGGSGGGGSEVQLVESGGGLVQPGGSLRLSCAASGRTFSSYTMGWFRQAPGKEREFVAAISWSGGRTYYADSVKGRFTISRDNSKNTVYLQMNSLRPEDTAVYYCAAYRRRRASSNRGLWDYWGQGTLVTVSSA

SEQ ID NO: 189 - protein, 279 aa, Artificial Sequence
  Amino acid sequence
EVQLVESGGGLVQPGGSLRLSCAASGSIFSINAMGWYRQAPGKQRELVAAISSGGSTYYADSVKGRFTISRDNSKNTVYLQMNSLRPEDTAVYYCNAAVDASRGLPYELYYYWGQGTLVTVSSGGGGSGGGGSGGGGSGGGGSGGGGSGGGGSGGGGSEVQLVESGGGLVQPGGSLRLSCAASGSTFIINVVRWYRRAPGKQRELVATISSGGNANYVDSVRGRFTISRDNSKNTVYLQMNSLRPEDTAVYYCNVPTTHYGGVYYGPYWGQGTLVTVSS

SEQ ID NO: 190 - protein, 435 aa, Artificial Sequence
  Amino acid sequence
EVQLVESGGGLVQPGGSLRLSCAASGSIFSINAMGWYRQAPGKQRELVAAISSGGSTYYADSVKGRFTISRDNSKNTVYLQMNSLRPEDTAVYYCNAAVDASRGLPYELYYYWGQGTLVTVSSGGGGSGGGGSGGGGSGGGGSGGGGSGGGGSGGGGSEVQLVESGGGLVQPGGSLRLSCAASGSTFIINVVRWYRRAPGKQRELVATISSGGNANYVDSVRGRFTISRDNSKNTVYLQMNSLRPEDTAVYYCNVPTTHYGGVYYGPYWGQGTLVTVSSGGGGSGGGGSGGGGSGGGGSGGGGSGGGGSGGGGSEVQLVESGGGLVQPGGSLRLSCAASGSTFIINVVRWYRRAPGKQRELVATISSGGNANYVDSVRGRFTISRDNSKNTVYLQMNSLRPEDTAVYYCNVPTTHYGGVYYGPYWGQGTLVTVSS

SEQ ID NO: 191 - protein, 282 aa, Artificial Sequence
  Amino acid sequence
EVQLVESGGGLVQPGGSLRLSCAASGSIFSINAMGWYRQAPGKQRELVAAISSGGSTYYADSVKGRFTISRDNSKNTVYLQMNSLRPEDTAVYYCNAAVDASRGLPYELYYYWGQGTLVTVSSGGGGSGGGGSGGGGSGGGGSGGGGSGGGGSGGGGSEVQLVESGGGLVQPGGSLRLSCAASGRTFSSYTMGWFRQAPGKEREFVAAISWSGGRTYYADSVKGRFTISRDNSKNTVYLQMNSLRPEDTAVYYCAAYRRRRASSNRGLWDYWGQGTLVTVSS

SEQ ID NO: 192 - protein, 434 aa, Artificial Sequence
  Amino acid sequence
EVQLVESGGGVVQPGGSLRLSCAASGFAFSAAYMSWVRQAPGKGLEWVSSISDDGSKTYYADSVKGRFTISRDNSKNTVYLQMNSLRPEDTALYYCNTGYGATTTRPGRYWGQGTLVTVSSGGGGSGGGGSGGGGSGGGGSGGGGSGGGGSGGGGSEVQLVESGGGVVQPGGSLRLSCAASGSTFIINVVRWYRRAPGKQRELVATISSGGNANYVDSVRGRFTISRDNSKNTVYLQMNSLRPEDTALYYCNVPTTHYGGVYYGPYWGQGTLVTVSSGGGGSGGGGSGGGGSGGGGSGGGGSGGGGSGGGGSEVQLVESGGGVVQPGGSLRLSCAASGSTFIINVVRWYRRAPGKQRELVATISSGGNANYVDSVRGRFTISRDNSKNTVYLQMNSLRPEDTALYYCNVPTTHYGGVYYGPYWGQGTLVTVSSA

SEQ ID NO: 193 - protein, 116 aa, Artificial Sequence
  Amino acid sequence
EVQLVESGGGLVQPGNSLRLSCAASGFTFSSFGMSWVRQAPGKGLEWVSSISGSGSDTLYADSVKGRFTISRDNAKTTLYLQMNSLRPEDTAVYYCTIGGSLSRSSQGTLVTVKSA

SEQ ID NO: 194 - protein, 155 aa, Artificial Sequence
  Amino acid sequence
EVQLVESGGGLVQPGGSLRLSCAASGFAFSAAYMSWVRQAPGKGLEWVSSISDDGSKTYYADSVKGRFTISRDNSKNTVYLQMNSLRPEDTAVYYCNTGYGATTTRPGRYWGQGTLVTVSSAAADYKDHDGDYKDHDIDYKDDDDKGAAHHHHHH

SEQ ID NO: 195 - protein, 162 aa, Artificial Sequence
  Amino acid sequence
EVQLVESGGGLVQPGGSLRLSCAASGFTLAYYSIGWFRQAPGKEREGVSCISSGIDGSTYYADSVKGRFTISRDNAKNTMYLQMNNLKPEDTGVYYCAADPSHYYSEYDCGYYGMDYWGKGTLVTVSSGAADYKDHDGDYKDHDIDYKDDDDKGAAHHHHHH

SEQ ID NO: 196 - protein, 312 aa, Artificial Sequence
  Amino acid sequence
EVQLVESGGGLVQPGGSLRLSCAASGRTFSSYAMGWFRQAPGKEREFVAAISWSGGSTYYADSVKGRFTISRDNSKNTVYLQMNSLRPEDTAVYYCTAALAVYGPNRYRYGPVGEYNYWGQGTLVTVSSGGGGSGGGGSGGGGSGGGGSGGGGSGGGGSGGGGSEVQLVESGGGSVQAGGSLRLSCAASGSTFSRYSMNWYRQAPGKQREFVAGISVGRITNYAVSVRGRFTISRDNAEGTGYLQMNSLKPEDTAVYYCNAGGLQGYWGLGTLVTVSSGAADYKDHDGDYKDHDIDYKDDDDKGAAHHHHHH

SEQ ID NO: 197 - protein, 157 aa, Artificial Sequence
  Amino acid sequence
EVQLVESGGGLVQPGGSLRLSCAASGSIFSINAMGWYRQAPGKQRELVAAISSGGSTYYADSVKGRFTISRDNSKNTVYLQMNSLRPEDTAVYYCNAAVDASRGLPYELYYYWGQGTLVTVSSAAADYKDHDGDYKDHDIDYKDDDDKGAAHHHHHH